European Patent Application EP 4 792 821 A2, published August 19, 2026. Title: Antiviral Polypeptide Membrane Fusion Inhibitor, and Preparation Method and Application Thereof. Applicant: Hangzhou Tianlong Pharmaceutical Co., Ltd. The sequence listing filed with the application follows.

SEQUENCE LISTING (136 sequences)

SEQ ID NO: 1 - protein, 32 aa, synthetic construct
  MOD_RES 1: note = Ac
  MOD_RES 32: note = NH2
FDASIEEVNRRIEESLRRIEESDRRLEVNKKA

SEQ ID NO: 2 - protein, 36 aa, synthetic construct
  MOD_RES 1: note = Ac
  MOD_RES 36: note = NH2
DDEFNQKINEVNEKIEEILKKIEESDRKLEESDKKA

SEQ ID NO: 3 - protein, 32 aa, synthetic construct
  MOD_RES 1: note = Ac
  MOD_RES 32: note = NH2
DEFDKKKIEEVNKKIEESLKKIEESDKKLEEV

SEQ ID NO: 4 - protein, 32 aa, synthetic construct
  MOD_RES 1: note = Ac
  MOD_RES 32: note = NH2
FDASLLKIEEEKKKIEELLKLHNESDKKLEEV

SEQ ID NO: 5 - protein, 36 aa, synthetic construct
  MOD_RES 1: note = Ac
  MOD_RES 36: note = NH2
WDEFDKKIEEVNKKIEESLKKIEESDKKLEEVNKKL

SEQ ID NO: 6 - protein, 36 aa, synthetic construct
  MOD_RES 1: note = Ac
  MOD_RES 36: note = NH2
ADAFRLEVNDASSKINESIEESLLSLEKLHNVNATA

SEQ ID NO: 7 - protein, 34 aa, synthetic construct
  MOD_RES 1: note = Ac
  MOD_RES 34: note = NH2
FDAFIQEINVNEDQSLEQSDELLLELHLLHSLLH

SEQ ID NO: 8 - protein, 36 aa, synthetic construct
  MOD_RES 1: note = Ac
  MOD_RES 36: note = NH2
FAEFNQKINQVNEKIEESLEEIRKSDEELHNVNATT

SEQ ID NO: 9 - protein, 42 aa, synthetic construct
  MOD_RES 1: note = Ac
  MOD_RES 42: note = NH2
  LIPID 42: note = Chol
WDEFDKKIEEVNKKIEESLKKIEESDKKLEEVNKKLEAAAKK

SEQ ID NO: 10 - protein, 36 aa, synthetic construct
  MOD_RES 1: note = Ac
  MOD_RES 36: note = NH2
  LIPID 36: note = Chol
KIEEVNKKIEESLKKIEESDKKLEEVNKKLEAAAKK

SEQ ID NO: 11 - protein, 42 aa, synthetic construct
  MOD_RES 1: note = Ac
  MOD_RES 42: note = NH2
  LIPID 42: note = Chol
WDEFDKKIEEVNKKIEESLKKIEESDKKLEEVNKKLGSGSGK

SEQ ID NO: 12 - protein, 38 aa, synthetic construct
  MOD_RES 1: note = Ac
  MOD_RES 38: note = NH2
  LIPID 38: note = Chol
FDASIEEVNRRIEESLRRIEESDRRLEVNKKAGSGSGK

SEQ ID NO: 13 - protein, 35 aa, synthetic construct
  MOD_RES 1: note = Ac
  MOD_RES 35: note = NH2
  LIPID 35: note = Chol
WDEFDKKIEEVNKKIEESLKKIEESDKKLEAAAKK

SEQ ID NO: 14 - protein, 38 aa, synthetic construct
  MOD_RES 1: note = Ac
  MOD_RES 38: note = NH2
  LIPID 38: note = Chol
DEFDKKIEEVNKKIEESLKKIEESDKKLEEVNEAAAKK

SEQ ID NO: 15 - protein, 38 aa, synthetic construct
  MOD_RES 1: note = Ac
  MOD_RES 38: note = NH2
  LIPID 38: note = Chol
DEFDKKKIEEVNKKIEESLKKIEESDKKLEEVGSGSGK

SEQ ID NO: 16 - protein, 35 aa, synthetic construct
  MOD_RES 1: note = Ac
  MOD_RES 35: note = NH2
  LIPID 35: note = Chol
SDEFDKKIEEVNKKIEESLKKIEESDKKLEAAAKK

SEQ ID NO: 17 - protein, 34 aa, synthetic construct
  MOD_RES 1: note = Ac
  MOD_RES 34: note = NH2
  LIPID 34: note = Chol
DEFDKKIEEVNKKIEESLKKIEESDKKLEAAAKK

SEQ ID NO: 18 - protein, 38 aa, synthetic construct; identical to SEQ ID NO: 15
  MOD_RES 1: note = Ac
  MOD_RES 38: note = NH2
  LIPID 38: note = Chol

SEQ ID NO: 19 - protein, 32 aa, synthetic construct
  MOD_RES 1: note = Ac
  MOD_RES 32: note = NH2
  LIPID 32: note = Chol
FDASIEEVNRRIEESLRRIEESDRRLEAAAKK

SEQ ID NO: 20 - protein, 35 aa, synthetic construct
  MOD_RES 1: note = Ac
  MOD_RES 35: note = NH2
  LIPID 35: note = Chol
SDEFDKKIEEVNKKIEESLKKIEESDKKLGSGSGK

SEQ ID NO: 21 - protein, 37 aa, synthetic construct
  MOD_RES 1: note = Ac
  MOD_RES 37: note = NH2
  LIPID 37: note = Chol
DEFDKKIEEVNKKIEESLKKIEESDKKLEEVEAAAKK

SEQ ID NO: 22 - protein, 38 aa, synthetic construct
  MOD_RES 1: note = Ac
  MOD_RES 38: note = NH2
  LIPID 38: note = Chol
DEFDKKKIEEVNKKIEESLKKIEESDKKLEEVEAAAKK

SEQ ID NO: 23 - protein, 32 aa, synthetic construct
  MOD_RES 1: note = Ac
  MOD_RES 32: note = NH2
YDELVFDASQVNEKINQSLEKIRKSDELLHNV

SEQ ID NO: 24 - protein, 42 aa, synthetic construct
  MOD_RES 1: note = Ac
  MOD_RES 42: note = NH2
FDFDEFDASISQVNEKINESLAFIRLAFIRKSDELLEAAAKK

SEQ ID NO: 25 - protein, 38 aa, synthetic construct
  MOD_RES 1: note = Ac
  MOD_RES 38: note = NH2
  LIPID 38: note = Chol
YDELVFDASQVNEKINQSLEKIRKSDELLHNVGSGSGK

SEQ ID NO: 26 - protein, 42 aa, synthetic construct
  MOD_RES 1: note = Ac
  MOD_RES 42: note = NH2
  LIPID 42: note = Chol
FDEEISQVNEKINQSLAFIRKSDELLHNVNAGKSTTEAAAKK

SEQ ID NO: 27 - protein, 42 aa, synthetic construct
  MOD_RES 1: note = Ac
  MOD_RES 42: note = NH2
  LIPID 42: note = Chol
WDEFDASISQVNEKINQSLEEIRKSDELLHNVNAGLGSGSGK

SEQ ID NO: 28 - protein, 36 aa, synthetic construct
  MOD_RES 1: note = Ac
  MOD_RES 36: note = NH2
  LIPID 36: note = Chol
DEFDASISQVNEKINQSLEEIRKSDELLHNEAAAKK

SEQ ID NO: 29 - protein, 42 aa, synthetic construct
  MOD_RES 1: note = Ac
  MOD_RES 42: note = NH2
  LIPID 42: note = Chol
LVKKIDEFDASISQVNEKINQSLEEIRKSDELLHNVGSGSGK

SEQ ID NO: 30 - protein, 38 aa, synthetic construct
  MOD_RES 1: note = Ac
  MOD_RES 38: note = NH2
  LIPID 38: note = Chol
YDELVFDASQVNEKINQSLEKIRKSDELLHNVEAAAKK

SEQ ID NO: 31 - protein, 31 aa, synthetic construct
  MOD_RES 1: note = Ac
  MOD_RES 31: note = NH2
  LIPID 31: note = Chol
SDEQVNEKINQSLAFIRRIRKLLHNEAAAKK

SEQ ID NO: 32 - protein, 31 aa, synthetic construct
  MOD_RES 1: note = Ac
  MOD_RES 31: note = NH2
  LIPID 31: note = Chol
ILELVNKKIEQSLKFIEKSDKLLENEAAAKK

SEQ ID NO: 33 - protein, 31 aa, synthetic construct
  MOD_RES 1: note = Ac
  MOD_RES 31: note = NH2
  LIPID 31: note = Chol
SLEQVNKKINQSLKVNKKSDKLLENEAAAKK

SEQ ID NO: 34 - protein, 31 aa, synthetic construct
  MOD_RES 1: note = Ac
  MOD_RES 31: note = NH2
  LIPID 31: note = Chol
FDEEVNKKIEQSLKINQSLEEIRKSEAAAKK

SEQ ID NO: 35 - protein, 31 aa, synthetic construct
  MOD_RES 1: note = Ac
  MOD_RES 31: note = NH2
  LIPID 31: note = Chol
SISQVNEKINEIQSLEEKSDKLLKSEAAAKK

SEQ ID NO: 36 - protein, 31 aa, synthetic construct
  MOD_RES 1: note = Ac
  MOD_RES 31: note = NH2
  LIPID 31: note = Chol
VNKKIEEEKQSLKKQSDKIEESDENEAAAKK

SEQ ID NO: 37 - protein, 31 aa, synthetic construct
  MOD_RES 1: note = Ac
  MOD_RES 31: note = NH2
  LIPID 31: note = Chol
FDELVNKKIEKIEEVNKKSLKLLESEAAAKK

SEQ ID NO: 38 - protein, 41 aa, synthetic construct
  MOD_RES 1: note = Ac
  MOD_RES 41: note = NH2
  LIPID 41: note = Chol
WDEFDASISQVNEKINQSLEEIRKSDELLHNVNALEAAAKK

SEQ ID NO: 39 - protein, 39 aa, synthetic construct
  MOD_RES 1: note = Ac
  MOD_RES 39: note = NH2
  LIPID 39: note = Chol
WDEFDASISQNEKINQSLEEIRKSDELLHNNALEAAAKK

SEQ ID NO: 40 - protein, 40 aa, synthetic construct
  MOD_RES 1: note = Ac
  MOD_RES 40: note = NH2
  LIPID 40: note = Chol
WDEFDKKIEEVNKKIEESLKKIEESDKKLEEVNAEAAAKK

SEQ ID NO: 41 - protein, 39 aa, synthetic construct
  MOD_RES 1: note = Ac
  MOD_RES 39: note = NH2
  LIPID 39: note = Chol
WDEFDKKIEEVNKKIEESLKKIEESDKKLEEVNEAAAKK

SEQ ID NO: 42 - protein, 37 aa, synthetic construct
  MOD_RES 1: note = Ac
  MOD_RES 37: note = NH2
  LIPID 37: note = Chol
FDASIEEVNRRIEESLRRIEESDRRLEEVNAEAAAKK

SEQ ID NO: 43 - protein, 38 aa, synthetic construct
  MOD_RES 1: note = Ac
  MOD_RES 38: note = NH2
  LIPID 38: note = Chol
WDEFDASIEEVNRRIEESLRRIEESDRRLEEVEAAAKK

SEQ ID NO: 44 - protein, 38 aa, synthetic construct
  MOD_RES 1: note = Ac
  MOD_RES 38: note = NH2
  LIPID 38: note = Chol
WDEFDKKIEEVNKKIEESLKKIEESDKKLHNVEAAAKK

SEQ ID NO: 45 - protein, 37 aa, synthetic construct
  MOD_RES 1: note = Ac
  MOD_RES 37: note = NH2
  LIPID 37: note = Chol
WDEFDASISQVNEKINQSLEEIRKSDELLHNEAAAKK

SEQ ID NO: 46 - protein, 34 aa, synthetic construct
  MOD_RES 1: note = Ac
  MOD_RES 34: note = NH2
FEVNRRRIEQSLEKSLESLEEEEHSDKKLHNELH

SEQ ID NO: 47 - protein, 42 aa, synthetic construct
  MOD_RES 1: note = Ac
  MOD_RES 42: note = NH2
SLEQVNKINKKIDKIEESLKKIEESDKKSLEVNKKLEAAAKK

SEQ ID NO: 48 - protein, 42 aa, synthetic construct
  MOD_RES 1: note = Ac
  MOD_RES 42: note = NH2
SLEQVNKINEKINKISQSLKKIEESDKKSDEVNAGLEAAAKK

SEQ ID NO: 49 - protein, 42 aa, synthetic construct
  MOD_RES 1: note = Ac
  MOD_RES 42: note = NH2
SLEQVNKKIEQSLESLKKSDKINQSLEEVNKSDELLEAAAKK

SEQ ID NO: 50 - protein, 42 aa, synthetic construct
  MOD_RES 1: note = Ac
  MOD_RES 42: note = NH2
SLEQVNEKINQSLAFIRKSDEINQSDEEVNKSDELLEAAAKK

SEQ ID NO: 51 - protein, 36 aa, synthetic construct
  MOD_RES 1: note = Ac
  MOD_RES 36: note = NH2
SDELVNKKIEFDKKINQSLKKIEESDKKKLEAAAKK

SEQ ID NO: 52 - protein, 32 aa, synthetic construct; identical to SEQ ID NO: 1

SEQ ID NO: 53 - protein, 36 aa, synthetic construct; identical to SEQ ID NO: 2

SEQ ID NO: 54 - protein, 32 aa, synthetic construct; identical to SEQ ID NO: 3

SEQ ID NO: 55 - protein, 32 aa, synthetic construct; identical to SEQ ID NO: 4

SEQ ID NO: 56 - protein, 36 aa, synthetic construct; identical to SEQ ID NO: 5

SEQ ID NO: 57 - protein, 36 aa, synthetic construct; identical to SEQ ID NO: 6

SEQ ID NO: 58 - protein, 34 aa, synthetic construct; identical to SEQ ID NO: 7

SEQ ID NO: 59 - protein, 36 aa, synthetic construct; identical to SEQ ID NO: 8

SEQ ID NO: 60 - protein, 36 aa, synthetic construct; identical to SEQ ID NO: 5

SEQ ID NO: 61 - protein, 30 aa, synthetic construct
KIEEVNKKIEESLKKIEESDKKLEEVNKKL

SEQ ID NO: 62 - protein, 36 aa, synthetic construct; identical to SEQ ID NO: 5

SEQ ID NO: 63 - protein, 32 aa, synthetic construct; identical to SEQ ID NO: 1

SEQ ID NO: 64 - protein, 29 aa, synthetic construct
WDEFDKKIEEVNKKIEESLKKIEESDKKL

SEQ ID NO: 65 - protein, 32 aa, synthetic construct
DEFDKKIEEVNKKIEESLKKIEESDKKLEEVN

SEQ ID NO: 66 - protein, 32 aa, synthetic construct; identical to SEQ ID NO: 3

SEQ ID NO: 67 - protein, 29 aa, synthetic construct
SDEFDKKIEEVNKKIEESLKKIEESDKKL

SEQ ID NO: 68 - protein, 28 aa, synthetic construct
DEFDKKIEEVNKKIEESLKKIEESDKKL

SEQ ID NO: 69 - protein, 32 aa, synthetic construct; identical to SEQ ID NO: 3

SEQ ID NO: 70 - protein, 26 aa, synthetic construct
FDASIEEVNRRIEESLRRIEESDRRL

SEQ ID NO: 71 - protein, 29 aa, synthetic construct
SDEFDKKIEEVNKKIEESLKKIEESDKKL

SEQ ID NO: 72 - protein, 31 aa, synthetic construct
DEFDKKIEEVNKKIEESLKKIEESDKKLEEV

SEQ ID NO: 73 - protein, 32 aa, synthetic construct; identical to SEQ ID NO: 3

SEQ ID NO: 74 - protein, 32 aa, synthetic construct; identical to SEQ ID NO: 23

SEQ ID NO: 75 - protein, 36 aa, synthetic construct
FDFDEFDASISQVNEKINESLAFIRLAFIRKSDELL

SEQ ID NO: 76 - protein, 32 aa, synthetic construct; identical to SEQ ID NO: 23

SEQ ID NO: 77 - protein, 36 aa, synthetic construct
FDEEISQVNEKINQSLAFIRKSDELLHNVNAGKSTT

SEQ ID NO: 78 - protein, 36 aa, synthetic construct
WDEFDASISQVNEKINQSLEEIRKSDELLHNVNAGL

SEQ ID NO: 79 - protein, 30 aa, synthetic construct
DEFDASISQVNEKINQSLEEIRKSDELLHN

SEQ ID NO: 80 - protein, 36 aa, synthetic construct
LVKKIDEFDASISQVNEKINQSLEEIRKSDELLHNV

SEQ ID NO: 81 - protein, 32 aa, synthetic construct; identical to SEQ ID NO: 23

SEQ ID NO: 82 - protein, 25 aa, synthetic construct
SDEQVNEKINQSLAFIRRIRKLLHN

SEQ ID NO: 83 - protein, 25 aa, synthetic construct
ILELVNKKIEQSLKFIEKSDKLLEN

SEQ ID NO: 84 - protein, 25 aa, synthetic construct
SLEQVNKKINQSLKVNKKSDKLLEN

SEQ ID NO: 85 - protein, 25 aa, synthetic construct
FDEEVNKKIEQSLKINQSLEEIRKS

SEQ ID NO: 86 - protein, 25 aa, synthetic construct
SISQVNEKINEIQSLEEKSDKLLKS

SEQ ID NO: 87 - protein, 25 aa, synthetic construct
VNKKIEEEKQSLKKQSDKIEESDEN

SEQ ID NO: 88 - protein, 25 aa, synthetic construct
FDELVNKKIEKIEEVNKKSLKLLES

SEQ ID NO: 89 - protein, 35 aa, synthetic construct
WDEFDASISQVNEKINQSLEEIRKSDELLHNVNAL

SEQ ID NO: 90 - protein, 33 aa, synthetic construct
WDEFDASISQNEKINQSLEEIRKSDELLHNNAL

SEQ ID NO: 91 - protein, 34 aa, synthetic construct
WDEFDKKIEEVNKKIEESLKKIEESDKKLEEVNA

SEQ ID NO: 92 - protein, 33 aa, synthetic construct
WDEFDKKIEEVNKKIEESLKKIEESDKKLEEVN

SEQ ID NO: 93 - protein, 31 aa, synthetic construct
FDASIEEVNRRIEESLRRIEESDRRLEEVNA

SEQ ID NO: 94 - protein, 32 aa, synthetic construct
WDEFDASIEEVNRRIEESLRRIEESDRRLEEV

SEQ ID NO: 95 - protein, 32 aa, synthetic construct
WDEFDKKIEEVNKKIEESLKKIEESDKKLHNV

SEQ ID NO: 96 - protein, 31 aa, synthetic construct
WDEFDASISQVNEKINQSLEEIRKSDELLHN

SEQ ID NO: 97 - protein, 34 aa, synthetic construct; identical to SEQ ID NO: 46

SEQ ID NO: 98 - protein, 36 aa, synthetic construct
SLEQVNKINKKIDKIEESLKKIEESDKKSLEVNKKL

SEQ ID NO: 99 - protein, 36 aa, synthetic construct
SLEQVNKINEKINKISQSLKKIEESDKKSDEVNAGL

SEQ ID NO: 100 - protein, 36 aa, synthetic construct
SLEQVNKKIEQSLESLKKSDKINQSLEEVNKSDELL

SEQ ID NO: 101 - protein, 36 aa, synthetic construct
SLEQVNEKINQSLAFIRKSDEINQSDEEVNKSDELL

SEQ ID NO: 102 - protein, 30 aa, synthetic construct
SDELVNKKIEFDKKINQSLKKIEESDKKKL

SEQ ID NO: 103 - protein, 53 aa, synthetic construct
  MOD_RES 1: note = Z1
  MOD_RES 53: note = Z3-Z2
  VARIANT 2..3: note = J represents acidic amino acids
  VARIANT 9..10: note = J represents acidic amino acids
  VARIANT 16..17: note = J represents acidic amino acids
  VARIANT 22..23: note = J represents acidic amino acids
  VARIANT 30..31: note = J represents acidic amino acids
  VARIANT 37..38: note = J represents acidic amino acids
  VARIANT 44..45: note = J represents acidic amino acids
  VARIANT 6..7: note = O represents basic amino acids
  VARIANT 13..14: note = O represents basic amino acids
  VARIANT 20..21: note = O represents basic amino acids
  VARIANT 27..28: note = O represents basic amino acids
  VARIANT 34..35: note = O represents basic amino acids
  VARIANT 41..42: note = O represents basic amino acids
  VARIANT 48..49: note = O represents basic amino acids
WJJLVOOSJJFDOOIJJVNOOIJJSLOOIJJSDOOLJJVNOOLJJTNOOITTI

SEQ ID NO: 104 - protein, 5 aa, synthetic construct
EAAAK

SEQ ID NO: 105 - protein, 5 aa, synthetic construct
GSGSG

SEQ ID NO: 106 - protein, 36 aa, synthetic construct; identical to SEQ ID NO: 6
  MOD_RES 1: note = R1
  MOD_RES 36: note = R2-R3

SEQ ID NO: 107 - protein, 34 aa, synthetic construct; identical to SEQ ID NO: 7
  MOD_RES 1: note = R1
  MOD_RES 34: note = R2-R3

SEQ ID NO: 108 - protein, 36 aa, synthetic construct; identical to SEQ ID NO: 8
  MOD_RES 1: note = R1
  MOD_RES 36: note = R2-R3

SEQ ID NO: 109 - protein, 25 aa, synthetic construct
  MOD_RES 1: note = R1
  MOD_RES 25: note = R2-R3
SDEQVNEKINQSLAFIRRIRKLLHN

SEQ ID NO: 110 - protein, 25 aa, synthetic construct
  MOD_RES 1: note = R1
  MOD_RES 25: note = R2-R3
ILELVNKKIEQSLKFIEKSDKLLEN

SEQ ID NO: 111 - protein, 25 aa, synthetic construct
  MOD_RES 1: note = R1
  MOD_RES 25: note = R2-R3
SLEQVNKKINQSLKVNKKSDKLLEN

SEQ ID NO: 112 - protein, 25 aa, synthetic construct
  MOD_RES 1: note = R1
  MOD_RES 25: note = R2-R3
FDEEVNKKIEQSLKINQSLEEIRKS

SEQ ID NO: 113 - protein, 25 aa, synthetic construct
  MOD_RES 1: note = R1
  MOD_RES 25: note = R2-R3
SISQVNEKINEIQSLEEKSDKLLKS

SEQ ID NO: 114 - protein, 25 aa, synthetic construct
  MOD_RES 1: note = R1
  MOD_RES 25: note = R2-R3
VNKKIEEEKQSLKKQSDKIEESDEN

SEQ ID NO: 115 - protein, 25 aa, synthetic construct
  MOD_RES 1: note = R1
  MOD_RES 25: note = R2-R3
FDELVNKKIEKIEEVNKKSLKLLES

SEQ ID NO: 116 - protein, 34 aa, synthetic construct; identical to SEQ ID NO: 46
  MOD_RES 1: note = R1
  MOD_RES 34: note = R2-R3

SEQ ID NO: 117 - protein, 36 aa, synthetic construct; identical to SEQ ID NO: 98
  MOD_RES 1: note = R1
  MOD_RES 36: note = R2-R3

SEQ ID NO: 118 - protein, 36 aa, synthetic construct; identical to SEQ ID NO: 99
  MOD_RES 1: note = R1
  MOD_RES 36: note = R2-R3

SEQ ID NO: 119 - protein, 36 aa, synthetic construct; identical to SEQ ID NO: 100
  MOD_RES 1: note = R1
  MOD_RES 36: note = R2-R3

SEQ ID NO: 120 - protein, 36 aa, synthetic construct; identical to SEQ ID NO: 101
  MOD_RES 1: note = R1
  MOD_RES 36: note = R2-R3

SEQ ID NO: 121 - protein, 30 aa, synthetic construct; identical to SEQ ID NO: 102
  MOD_RES 1: note = R1
  MOD_RES 30: note = R2-R3

SEQ ID NO: 122 - protein, 38 aa, synthetic construct
  VARIANT 1: note = X is D or absent.
  VARIANT 2: note = X is E or absent.
  VARIANT 3: note = X is W, F, D, S or absent.
  VARIANT 4: note = X is D or absent.
  VARIANT 5: note = X is E, A, K or absent.
  VARIANT 6: note = X is F, S or absent.
  VARIANT 7: note = X is D, N, L or absent.
  VARIANT 8: note = X is K, Q, L, or absent.
  VARIANT 9: note = X is K or absent.
  VARIANT 11: note = X is E or N.
  VARIANT 13: note = X is V or E.
  VARIANT 14: note = X is N or K.
  VARIANT 15: note = X is K, R or E.
  VARIANT 16: note = X is K or R
  VARIANT 20: note = X is S, I or L.
  VARIANT 22: note = X is K or R.
  VARIANT 23: note = X is K or R.
  VARIANT 24: note = X is I or H.
  VARIANT 25: note = X is E or N.
  VARIANT 29: note = X is K or R.
  VARIANT 30: note = X is K or R.
  VARIANT 32: note = X is E or absent.
  VARIANT 33: note = X is E, V or absent.
  VARIANT 34: note = X is V, N, S or absent.
  VARIANT 35: note = X is N, K, D or absent.
  VARIANT 36: note = X is K or absent.
  VARIANT 37: note = X is K, A or absent.
  VARIANT 38: note = X is L, A or absent.
XXXXXXXXXIXEXXXXIEEXLXXXXESDXXLXXXXXXX

SEQ ID NO: 123 - protein, 50 aa, synthetic construct
  VARIANT 1: note = X is F, W , D, L or Y.
  VARIANT 2: note = X is V or absent.
  VARIANT 3: note = X is K or absent.
  VARIANT 4: note = X is D, K or absent.
  VARIANT 5: note = X is F, I or absent.
  VARIANT 6: note = X is D or absent.
  VARIANT 8: note = X is L or absent.
  VARIANT 9: note = X is V or absent.
  VARIANT 10: note = X is F or absent.
  VARIANT 11: note = X is E or D.
  VARIANT 12: note = X is A or I.
  VARIANT 13: note = X is S or absent.
  VARIANT 14: note = X is I or absent.
  VARIANT 23: note = X is E or Q.
  VARIANT 26: note = X is A or E.
  VARIANT 27: note = X is F, E or K.
  VARIANT 30: note = X is L or absent.
  VARIANT 31: note = X is A or absent.
  VARIANT 32: note = X is F or absent.
  VARIANT 33: note = X is I or absent.
  VARIANT 34: note = X is R or absent.
  VARIANT 41: note = X is H or absent.
  VARIANT 42: note = X is N or absent.
  VARIANT 43: note = X is V or absent.
  VARIANT 44: note = X is N or absent.
  VARIANT 45: note = X is A or absent.
  VARIANT 46: note = X is G or absent.
  VARIANT 47: note = X is K, L or absent.
  VARIANT 48: note = X is S or absent.
  VARIANT 49: note = X is T or absent.
  VARIANT 50: note = X is T or absent.
XXXXXXEXXXXXXXSQVNEKINXSLXXIRXXXXXKSDELLXXXXXXXXXX

SEQ ID NO: 124 - protein, 34 aa, synthetic construct
  VARIANT 1: note = X is W or F.
  VARIANT 2: note = X is D or absent.
  VARIANT 3: note = X is E or absent.
  VARIANT 4: note = X is F or absent.
  VARIANT 6: note = X is K or A.
  VARIANT 7: note = X is K or S.
  VARIANT 13: note = X is K or R.
  VARIANT 14: note = X is K or R.
  VARIANT 20: note = X is K or R.
  VARIANT 21: note = X is K or R.
  VARIANT 27: note = X is K or R.
  VARIANT 28: note = X is K or R.
  VARIANT 30: note = X is E or H.
  VARIANT 31: note = X is E or N
  VARIANT 33: note = X is N or absent.
  VARIANT 34: note = X is A or absent.
XXXXDXXIEEVNXXIEESLXXIEESDXXLXXVXX

SEQ ID NO: 125 - protein, 35 aa, synthetic construct
  VARIANT 11: note = X is V or absent.
  VARIANT 32: note = X is V, N or absent.
  VARIANT 33: note = X is N, A or absent.
  VARIANT 34: note = X is A, L or absent.
  VARIANT 35: note = X is L or absent.
WDEFDASISQXNEKINQSLEEIRKSDELLHNXXXX

SEQ ID NO: 126 - protein, 38 aa, synthetic construct; identical to SEQ ID NO: 122
  MOD_RES 1: note = R1
  MOD_RES 38: note = R2-R3
  VARIANT 1: note = X is D or absent.
  VARIANT 2: note = X is E or absent.
  VARIANT 3: note = X is W, F, D, S or absent.
  VARIANT 4: note = X is D or absent.
  VARIANT 5: note = X is E, A, K or absent.
  VARIANT 6: note = X is F, S or absent.
  VARIANT 7: note = X is D, N, L or absent.
  VARIANT 8: note = X is K, Q, L or absent.
  VARIANT 9: note = X is K or absent.
  VARIANT 11: note = X is E or N.
  VARIANT 13: note = X is V or E.
  VARIANT 14: note = X is N or K.
  VARIANT 15: note = X is K, R or E.
  VARIANT 16: note = X is K or R.
  VARIANT 20: note = X is S, I or L.
  VARIANT 22: note = X is K or R.
  VARIANT 23: note = X is K or R.
  VARIANT 24: note = X is I or H.
  VARIANT 25: note = X is E or N.
  VARIANT 29: note = X is K or R.
  VARIANT 30: note = X is K or R.
  VARIANT 32: note = X is E or absent.
  VARIANT 33: note = X is E, V or absent.
  VARIANT 34: note = X is V, N, S or absent.
  VARIANT 35: note = X is N, K, D or absent.
  VARIANT 36: note = X is K or absent.
  VARIANT 37: note = X is K, A or absent.
  VARIANT 38: note = X is L, A or absent.

SEQ ID NO: 127 - protein, 50 aa, synthetic construct
  VARIANT 1: note = X is F, W, D, L or Y.
  VARIANT 2: note = X is V or absent.
  VARIANT 3: note = X is K or absent.
  VARIANT 4: note = X is D, K or absent.
  VARIANT 5: note = X is F, I or absent.
  VARIANT 6: note = X is D or absent.
  VARIANT 8: note = X is L or absent.
  VARIANT 9: note = X is V or absent.
  VARIANT 10: note = X is F or absent.
  VARIANT 11: note = X is E or D.
  VARIANT 12: note = X is A or I.
  VARIANT 13: note = X is S or absent.
  VARIANT 14: note = X is I or absent.
  VARIANT 23: note = X is E or Q.
  VARIANT 26: note = X is A or E.
  VARIANT 27: note = X is F, E or K.
  VARIANT 30: note = X is L or absent.
  VARIANT 31: note = X is A or absent.
  VARIANT 32: note = X is F or absent.
  VARIANT 33: note = X is I or absent.
  VARIANT 34: note = X is R or absent.
  VARIANT 41: note = X is H or absent.
  VARIANT 42: note = X is N or absent.
  VARIANT 43: note = X is V or absent.
  VARIANT 44: note = X is N or absent.
  VARIANT 45: note = X is A or absent.
  VARIANT 46: note = X is G or absent.
  VARIANT 47: note = X is K, L or absent.
  VARIANT 48: note = X is S or absent.
  VARIANT 49: note = X is T or absent.
  VARIANT 50: note = X is T or absent.
  MOD_RES 1: note = R1
  MOD_RES 50: note = R2-R3
XXXXXXEXXIXXXXSQVNEKINXSLXXIRXXXXXKSDELLXXXXXXXXXX

SEQ ID NO: 128 - protein, 34 aa, synthetic construct; identical to SEQ ID NO: 124
  VARIANT 1: note = X is W or F.
  VARIANT 2: note = X is D or absent.
  VARIANT 3: note = X is E or absent.
  VARIANT 4: note = X is F or absent.
  VARIANT 6: note = X is K or A.
  VARIANT 7: note = X is K or S.
  VARIANT 13: note = X is K or R.
  VARIANT 14: note = X is K or R.
  VARIANT 20: note = X is K or R.
  VARIANT 21: note = X is K or R.
  VARIANT 27: note = X is K or R.
  VARIANT 28: note = X is K or R.
  VARIANT 30: note = X is E or H.
  VARIANT 31: note = X is E or N.
  VARIANT 33: note = X is N or absent.
  VARIANT 34: note = X is A or absent.
  MOD_RES 1: note = R1
  MOD_RES 34: note = R2-R3

SEQ ID NO: 129 - protein, 35 aa, synthetic construct; identical to SEQ ID NO: 125
  MOD_RES 1: note = R1
  MOD_RES 35: note = R2-R3
  VARIANT 11: note = X is V or absent.
  VARIANT 32: note = X is V, N or absent.
  VARIANT 33: note = X is N, A or absent.
  VARIANT 34: note = X is A, L or absent.
  VARIANT 35: note = X is L or absent.

SEQ ID NO: 130 - protein, 31 aa, synthetic construct
  MOD_RES 1: note = Ac
  MOD_RES 31: note = NH2
  LIPID 31: note = Chol
SLEQVNKKIEQSLKFIEKSDKLLENGSGSGK

SEQ ID NO: 131 - protein, 29 aa, synthetic construct
  MOD_RES 1: note = Ac
  MOD_RES 29: note = NH2
IEQVNKKIEQSLKFIEKSDKLLENVNKGK

SEQ ID NO: 132 - protein, 35 aa, synthetic construct
  MOD_RES 1: note = Ac
  MOD_RES 35: note = NH2
  LIPID 35: note = Chol
IEEVNKKIEESLKKIEESDKKLEEVNKKKEAAAKK

SEQ ID NO: 133 - protein, 36 aa, synthetic construct
  LIPID 36: note = Chol
  MOD_RES 1: note = Ac
  MOD_RES 36: note = NH2
IEQVNKKIEQSLKFIEKSDKLLENVNKGKCEAAAKK

SEQ ID NO: 134 - protein, 36 aa, synthetic construct
  MOD_RES 1: note = Ac
  MOD_RES 36: note = NH2
  LIPID 36: note = Chol
LEQVNKKIEQSLKFIEKSDKLLENVNKGKCEAAAKK

SEQ ID NO: 135 - protein, 35 aa, synthetic construct
  MOD_RES 1: note = Ac
  MOD_RES 35: note = NH2
VFPSDEFDASISQVNEKINQSLAAIRKSDELLHNV

SEQ ID NO: 136 - protein, 42 aa, synthetic construct
  MOD_RES 1: note = Ac
  MOD_RES 42: note = NH2
  LIPID 42: note = Chol
FDASISQVNEKINQSLAFIRKSDELLHNVNAGKSTTEAAAKK